European Patent Specification EP 3 988 656 B1, published September 18, 2024. Title: USING NUCLEOSOME INTERACTING PROTEIN DOMAINS TO ENHANCE TARGETED GENOME MODIFICATION. Applicant: SIGMA-ALDRICH CO. LLC. The sequence listing filed with the application follows.

SEQUENCE LISTING (79 sequences)

SEQ ID NO: 1 - protein, 6 aa, Artificial Sequence
  SYNTHESIZED
LEGGGS

SEQ ID NO: 2 - protein, 4 aa, Artificial Sequence
  SYNTHESIZED
TGSG

SEQ ID NO: 3 - protein, 8 aa, Artificial Sequence
  SYNTHESIZED
GGSGGGSG

SEQ ID NO: 4 - protein, 20 aa, Artificial Sequence
  SYNTHESIZED
  MISC_FEATURE (6)..(20): can be either absent or present
GGGGSGGGGSGGGGSGGGGS

SEQ ID NO: 5 - protein, 8 aa, Artificial Sequence
  SYNTHESIZED
  MISC_FEATURE (7)..(8): can be either absent or present)
GGGGGGGG

SEQ ID NO: 6 - protein, 20 aa, Artificial Sequence
  SYNTHESIZED
  MISC_FEATURE (6)..(20): can be either absent or present
EAAAKEAAAKEAAAKEAAAK

SEQ ID NO: 7 - protein, 27 aa, Artificial Sequence
  SYNTHESIZED
  MISC_FEATURE (12)..(26): can be either absent or present
AEAAAKEAAAKEAAAKEAAAKEAAAKA

SEQ ID NO: 8 - protein, 5 aa, Artificial Sequence
  SYNTHESIZED
PAPAP

SEQ ID NO: 9 - protein, 16 aa, Artificial Sequence
  SYNTHESIZED
  MISC_FEATURE (13)..(16): can be either absent or present
APAPAPAPAPAPAPAP

SEQ ID NO: 10 - protein, 7 aa, Artificial Sequence
  SYNTHESIZED
PKKKRKV

SEQ ID NO: 11 - protein, 7 aa, Artificial Sequence
  SYNTHESIZED
PKKKRRV

SEQ ID NO: 12 - protein, 16 aa, Artificial Sequence
  SYNTHESIZED
KRPAATKKAGQAKKKK

SEQ ID NO: 13 - protein, 11 aa, Artificial Sequence
  SYNTHESIZED
YGRKKRRQRRR

SEQ ID NO: 14 - protein, 9 aa, Artificial Sequence
  SYNTHESIZED
RKKRRQRRR

SEQ ID NO: 15 - protein, 9 aa, Artificial Sequence
  SYNTHESIZED
PAAKRVKLD

SEQ ID NO: 16 - protein, 11 aa, Artificial Sequence
  SYNTHESIZED
RQRRNELKRSP

SEQ ID NO: 17 - protein, 8 aa, Artificial Sequence
  SYNTHESIZED
VSRKRPRP

SEQ ID NO: 18 - protein, 8 aa, Artificial Sequence
  SYNTHESIZED
PPKKARED

SEQ ID NO: 19 - protein, 8 aa, Artificial Sequence
  SYNTHESIZED
PQPKKKPL

SEQ ID NO: 20 - protein, 12 aa, Artificial Sequence
  SYNTHESIZED
SALIKKKKKMAP

SEQ ID NO: 21 - protein, 7 aa, Artificial Sequence
  SYNTHESIZED
PKQKKRK

SEQ ID NO: 22 - protein, 10 aa, Artificial Sequence
  SYNTHESIZED
RKLKKKIKKL

SEQ ID NO: 23 - protein, 10 aa, Artificial Sequence
  SYNTHESIZED
REKKKFLKRR

SEQ ID NO: 24 - protein, 20 aa, Artificial Sequence
  SYNTHESIZED
KRKGDEVDGVDEVAKKKSKK

SEQ ID NO: 25 - protein, 17 aa, Artificial Sequence
  SYNTHESIZED
RKCLQAGMNLEARKTKK

SEQ ID NO: 26 - protein, 38 aa, Artificial Sequence
  SYNTHESIZED
NQSSNFGPMKGGNFGGRSSGPYGGGGQYFAKPRNQGGY

SEQ ID NO: 27 - protein, 42 aa, Artificial Sequence
  SYNTHESIZED
RMRIZFKNKGKDTAELRRRRVEVSVELRKAKKDEQILKRRNV

SEQ ID NO: 28 - protein, 20 aa, Artificial Sequence
  SYNTHESIZED
GRKKRRQRRRPPQPKKKRKV

SEQ ID NO: 29 - protein, 19 aa, Artificial Sequence
  SYNTHESIZED
PLSSIFSRIGDPPKKKRKV

SEQ ID NO: 30 - protein, 24 aa, Artificial Sequence
  SYNTHESIZED
GALFLGWLGAAGSTMGAPKKKRKV

SEQ ID NO: 31 - protein, 27 aa, Artificial Sequence
  SYNTHESIZED
GALFLGFLGAAGSTMGAWSQPKKKRKV

SEQ ID NO: 32 - protein, 21 aa, Artificial Sequence
  SYNTHESIZED
KETWWETWWTEWSQPKKKRKV

SEQ ID NO: 33 - protein, 11 aa, Artificial Sequence
  SYNTHESIZED
YARAAARQARA

SEQ ID NO: 34 - protein, 11 aa, Artificial Sequence
  SYNTHESIZED
THRLPRRRRRR

SEQ ID NO: 35 - protein, 11 aa, Artificial Sequence
  SYNTHESIZED
GGRRARRRRRR

SEQ ID NO: 36 - protein, 12 aa, Artificial Sequence
  SYNTHESIZED
RRQRRTSKLMKR

SEQ ID NO: 37 - protein, 27 aa, Artificial Sequence
  SYNTHESIZED
GWTLNSAGYLLGKINLKALAALAKKIL

SEQ ID NO: 38 - protein, 33 aa, Artificial Sequence
  SYNTHESIZED
KALAWEAKLAKALAKALAKHLAKALAKALKCEA

SEQ ID NO: 39 - protein, 16 aa, Artificial Sequence
  SYNTHESIZED
RQIKIWFQNRRMKWKK

SEQ ID NO: 40 - protein, 84 aa, Homo sapiens
MGKGDPKKPRGKMSSYAFFVQTCREEHKKKHPDASVNFSEFSKKCSERWKTMSAKEKGKFEDMAKADKARYEREMKTYIPPKGE

SEQ ID NO: 41 - protein, 100 aa, Homo sapiens
MPKRKVSSAEGAAKEEPKRRSARLSAKPPAKVEAKPKKAAAKDKSSDKKVQTKGKRGAKGKQAEVANQETKEDLPAENGETKTEESPASDEAGEKEAKSD

SEQ ID NO: 42 - protein, 90 aa, Homo sapiens
MPKRKAEGDAKGDKAKVKDEPQRRSARLSAKPAPPKPEPKPKKAPAKKGEKVPKGKKGKADAGKEGNNPAENGDAKTDQAQKAEGAGDAK

SEQ ID NO: 43 - protein, 99 aa, Homo sapiens
MPKRKSPENTEGKDGSKVTKQEPTRRSARLSAKPAPPKPEPKPRKTSAKKEPGAKISRGAKGKKEEKQEAGKEGTAPSENGETKAEEAQKTESVDNEGE

SEQ ID NO: 44 - protein, 77 aa, Homo sapiens
MPKRKSPENTEGKDGSKVTKQEPTRRSARLSAKPAPPKPEPKPRKTSAKKEPGAKISRGAKGKKEEKQEAGKEGTEN

SEQ ID NO: 45 - protein, 80 aa, Homo sapiens
STDHPKYSDMIVAAIQAEKNRAGSSRQSIQKYIKSHYKVGENADSQIKLSIKRLVTTGVLKQTKGVGASGSFRLAKSDEP

SEQ ID NO: 46 - protein, 367 aa, Saccharomyces cerevisiae
LLNPTKRERKENYSIDNYYKDVLNTGRSSTPSHPRMPKPHVFHSHQLQPPQLKVLYEKERMWTAKKTGYVPTMDDVKAAYGDISDEEEKKQKLELLKLSVNNSQPLTEEEEKMKADWESEGFTNWNKLEFRKFITVSGKYGRNSIQAIARELAPGKTLEEVRAYAKAFWSNIERIEDYEKYLKIIENEEEKIKRVKMQQEALRRKLSEYKNPFFDLKLKHPPSSNNKRTYSEEEDRFILLMLFKYGLDRDDVYELVRDEIRDCPLFELDFYFRSRTPVELARRGNTLLQCLEKEFNAGIVLDDATKDRMKKEDENGKRIREEFADQTANEKENVDGVESKKAKIEDTSNVGTEQLVAEKIPENETTH

SEQ ID NO: 47 - protein, 269 aa, Saccharomyces cerevisiae
DMDSIGESEVRALYKAILKFGNLKEILDELIADGTLPVKSFEKYGETYDEMMEAAKDCVHEEEKNRKEILEKLEKHATAYRAKLKSGEIKAENQPKDNPLTRLSLKKREKKAVLFNFKGVKSLNAESLLSRVEDLKYLKNLINSNYKDDPLKFSLGNNTPKPVQNWSSNWTKEEDEKLLIGVFKYGYGSWTQIRDDPFLGITDKIFLNEVHNPVAKKSASSSDTTPTPSKKGKGITGSSKKVPGAIHLGRRVDYLLSFLRGGLNTKSPS

SEQ ID NO: 48 - DNA, 23 bp, Homo sapiens
agccgtgagtggagggagcgtgg

SEQ ID NO: 49 - DNA, 23 bp, Homo sapiens
agagggaggggttggactacagg

SEQ ID NO: 50 - DNA, 23 bp, Homo sapiens
cattcgccagtacgagcttgtgg

SEQ ID NO: 51 - DNA, 23 bp, Homo sapiens
ctttaatgcgctgacttgtgagg

SEQ ID NO: 52 - DNA, 23 bp, Homo sapiens
gtggcgcattgccacgaagcagg

SEQ ID NO: 53 - DNA, 23 bp, Homo sapiens
ttcttcttctgctcggactcagg

SEQ ID NO: 54 - DNA, 26 bp, Homo sapiens
tgctggaaaggggagaccaagggtga

SEQ ID NO: 55 - DNA, 26 bp, Homo sapiens
agagctacgagaaccagaagccgtga

SEQ ID NO: 56 - DNA, 26 bp, Homo sapiens
ttcccggcctcacccttggtctcccc

SEQ ID NO: 57 - DNA, 26 bp, Homo sapiens
ttggtctcccctttccagcattcgcc

SEQ ID NO: 58 - DNA, 26 bp, Homo sapiens
ttccagcattcgccagtacgagcttg

SEQ ID NO: 59 - DNA, 30 bp, Homo sapiens
gatcaacatgggagactcccacgtggacac

SEQ ID NO: 60 - DNA, 30 bp, Homo sapiens
agatacttcttcggccaccgcctcggacac

SEQ ID NO: 61 - protein, 1465 aa, Artificial Sequence
  SYNTHESIZED
MDKKYSIGLDIGTNSVGWAVITDEYKVPSKKFKVLGNTDRHSIKKNLIGALLFDSGETAEATRLKRTARRRYTRRKNRICYLQEIFSNEMAKVDDSFFHRLEESFLVEEDKKHERHPIFGNIVDEVAYHEKYPTIYHLRKKLVDSTDKADLRLIYLALAHMIKFRGHFLIEGDLNPDNSDVDKLFIQLVQTYNQLFEENPINASGVDAKAILSARLSKSRRLENLIAQLPGEKKNGLFGNLIALSLGLTPNFKSNFDLAEDAKLQLSKDTYDDDLDNLLAQIGDQYADLFLAAKNLSDAILLSDILRVNTEITKAPLSASMIKRYDEHHQDLTLLKALVRQQLPEKYKEIFFDQSKNGYAGYIDGGASQEEFYKFIKPILEKMDGTEELLVKLNREDLLRKQRTFDNGSIPHQIHLGELHAILRRQEDFYPFLKDNREKIEKILTFRIPYYVGPLARGNSRFAWMTRKSEETITPWNFEEVVDKGASAQSFIERMTNFDKNLPNEKVLPKHSLLYEYFTVYNELTKVKYVTEGMRKPAFLSGEQKKAIVDLLFKTNRKVTVKQLKEDYFKKIECFDSVEISGVEDRFNASLGTYHDLLKIIKDKDFLDNEENEDILEDIVLTLTLFEDREMIEERLKTYAHLFDDKVMKQLKRRRYTGWGRLSRKLINGIRDKQSGKTILDFLKSDGFANRNFMQLIHDDSLTFKEDIQKAQVSGQGDSLHEHIANLAGSPAIKKGILQTVKIVDELVKVMGHKPENIVIEMARENQTTQKGQKNSRERMKRIEEGIKELGSQILKEHPVENTQLQNEKLYLYYLQNGRDMYVDQELDINRLSDYDVDHIVPQSFIKDDSIDNKVLTRSDKNRGKSDNVPSEEVVKKMKNYWRQLLNAKLITQRKFDNLTKAERGGLSELDKAGFIKRQLVETRQITKHVAQILDSRMNTKYDENDKLIREVKVITLKSKLVSDFRKDFQFYKVREINNYHHAHDAYLNAVVGTALIKKYPKLESEFVYGDYKVYDVRKMIAKSEQEIGKATAKYFFYSNIMNFFKTEITLANGEIRKRPLIETNGETGEIVWDKGRDFATVRKVLSMPQVNIVKKTEVQTGGFSKESILPKRNSDKLIARKKDWDPKKYGGFDSPTVAYSVLVVAKVEKGKSKKLKSVKELLGITIMERSSFEKNPIDFLEAKGYKEVKKDLIIKLPKYSLFELENGRKRMLASAGELQKGNELALPSKYVNFLYLASHYEKLKGSPEDNEQKQLFVEQHKHYLDEIIEQISEFSKRVILADANLDKVLSAYNKHRDKPIREQAENIIHLFTLTNLGAPAAFKYFDTTIDRKRYTSTKEVLDATLIHQSITGLYETRIDLSQLGGDPKKKRKVLEGGGGSMGKGDPKKPRGKMSSYAFFVQTCREEHKKKHPDASVNFSEFSKKCSERWKTMSAKEKGKFEDMAKADKARYEREMKTYIPPKGE

SEQ ID NO: 62 - protein, 1481 aa, Artificial Sequence
  SYNTHESIZED
MDKKYSIGLDIGTNSVGWAVITDEYKVPSKKFKVLGNTDRHSIKKNLIGALLFDSGETAEATRLKRTARRRYTRRKNRICYLQEIFSNEMAKVDDSFFHRLEESFLVEEDKKHERHPIFGNIVDEVAYHEKYPTIYHLRKKLVDSTDKADLRLIYLALAHMIKFRGHFLIEGDLNPDNSDVDKLFIQLVQTYNQLFEENPINASGVDAKAILSARLSKSRRLENLIAQLPGEKKNGLFGNLIALSLGLTPNFKSNFDLAEDAKLQLSKDTYDDDLDNLLAQIGDQYADLFLAAKNLSDAILLSDILRVNTEITKAPLSASMIKRYDEHHQDLTLLKALVRQQLPEKYKEIFFDQSKNGYAGYIDGGASQEEFYKFIKPILEKMDGTEELLVKLNREDLLRKQRTFDNGSIPHQIHLGELHAILRRQEDFYPFLKDNREKIEKILTFRIPYYVGPLARGNSRFAWMTRKSEETITPWNFEEVVDKGASAQSFIERMTNFDKNLPNEKVLPKHSLLYEYFTVYNELTKVKYVTEGMRKPAFLSGEQKKAIVDLLFKTNRKVTVKQLKEDYFKKIECFDSVEISGVEDRFNASLGTYHDLLKIIKDKDFLDNEENEDILEDIVLTLTLFEDREMIEERLKTYAHLFDDKVMKQLKRRRYTGWGRLSRKLINGIRDKQSGKTILDFLKSDGFANRNFMQLIHDDSLTFKEDIQKAQVSGQGDSLHEHIANLAGSPAIKKGILQTVKIVDELVKVMGHKPENIVIEMARENQTTQKGQKNSRERMKRIEEGIKELGSQILKEHPVENTQLQNEKLYLYYLQNGRDMYVDQELDINRLSDYDVDHIVPQSFIKDDSIDNKVLTRSDKNRGKSDNVPSEEVVKKMKNYWRQLLNAKLITQRKFDNLTKAERGGLSELDKAGFIKRQLVETRQITKHVAQILDSRMNTKYDENDKLIREVKVITLKSKLVSDFRKDFQFYKVREINNYHHAHDAYLNAVVGTALIKKYPKLESEFVYGDYKVYDVRKMIAKSEQEIGKATAKYFFYSNIMNFFKTEITLANGEIRKRPLIETNGETGEIVWDKGRDFATVRKVLSMPQVNIVKKTEVQTGGFSKESILPKRNSDKLIARKKDWDPKKYGGFDSPTVAYSVLVVAKVEKGKSKKLKSVKELLGITIMERSSFEKNPIDFLEAKGYKEVKKDLIIKLPKYSLFELENGRKRMLASAGELQKGNELALPSKYVNFLYLASHYEKLKGSPEDNEQKQLFVEQHKHYLDEIIEQISEFSKRVILADANLDKVLSAYNKHRDKPIREQAENIIHLFTLTNLGAPAAFKYFDTTIDRKRYTSTKEVLDATLIHQSITGLYETRIDLSQLGGDPKKKRKVLEGGGGSMPKRKVSSAEGAAKEEPKRRSARLSAKPPAKVEAKPKKAAAKDKSSDKKVQTKGKRGAKGKQAEVANQETKEDLPAENGETKTEESPASDEAGEKEAKSD

SEQ ID NO: 63 - protein, 1471 aa, Artificial Sequence
  SYNTHESIZED
MDKKYSIGLDIGTNSVGWAVITDEYKVPSKKFKVLGNTDRHSIKKNLIGALLFDSGETAEATRLKRTARRRYTRRKNRICYLQEIFSNEMAKVDDSFFHRLEESFLVEEDKKHERHPIFGNIVDEVAYHEKYPTIYHLRKKLVDSTDKADLRLIYLALAHMIKFRGHFLIEGDLNPDNSDVDKLFIQLVQTYNQLFEENPINASGVDAKAILSARLSKSRRLENLIAQLPGEKKNGLFGNLIALSLGLTPNFKSNFDLAEDAKLQLSKDTYDDDLDNLLAQIGDQYADLFLAAKNLSDAILLSDILRVNTEITKAPLSASMIKRYDEHHQDLTLLKALVRQQLPEKYKEIFFDQSKNGYAGYIDGGASQEEFYKFIKPILEKMDGTEELLVKLNREDLLRKQRTFDNGSIPHQIHLGELHAILRRQEDFYPFLKDNREKIEKILTFRIPYYVGPLARGNSRFAWMTRKSEETITPWNFEEVVDKGASAQSFIERMTNFDKNLPNEKVLPKHSLLYEYFTVYNELTKVKYVTEGMRKPAFLSGEQKKAIVDLLFKTNRKVTVKQLKEDYFKKIECFDSVEISGVEDRFNASLGTYHDLLKIIKDKDFLDNEENEDILEDIVLTLTLFEDREMIEERLKTYAHLFDDKVMKQLKRRRYTGWGRLSRKLINGIRDKQSGKTILDFLKSDGFANRNFMQLIHDDSLTFKEDIQKAQVSGQGDSLHEHIANLAGSPAIKKGILQTVKIVDELVKVMGHKPENIVIEMARENQTTQKGQKNSRERMKRIEEGIKELGSQILKEHPVENTQLQNEKLYLYYLQNGRDMYVDQELDINRLSDYDVDHIVPQSFIKDDSIDNKVLTRSDKNRGKSDNVPSEEVVKKMKNYWRQLLNAKLITQRKFDNLTKAERGGLSELDKAGFIKRQLVETRQITKHVAQILDSRMNTKYDENDKLIREVKVITLKSKLVSDFRKDFQFYKVREINNYHHAHDAYLNAVVGTALIKKYPKLESEFVYGDYKVYDVRKMIAKSEQEIGKATAKYFFYSNIMNFFKTEITLANGEIRKRPLIETNGETGEIVWDKGRDFATVRKVLSMPQVNIVKKTEVQTGGFSKESILPKRNSDKLIARKKDWDPKKYGGFDSPTVAYSVLVVAKVEKGKSKKLKSVKELLGITIMERSSFEKNPIDFLEAKGYKEVKKDLIIKLPKYSLFELENGRKRMLASAGELQKGNELALPSKYVNFLYLASHYEKLKGSPEDNEQKQLFVEQHKHYLDEIIEQISEFSKRVILADANLDKVLSAYNKHRDKPIREQAENIIHLFTLTNLGAPAAFKYFDTTIDRKRYTSTKEVLDATLIHQSITGLYETRIDLSQLGGDPKKKRKVLEGGGGSMPKRKAEGDAKGDKAKVKDEPQRRSARLSAKPAPPKPEPKPKKAPAKKGEKVPKGKKGKADAGKEGNNPAENGDAKTDQAQKAEGAGDAK

SEQ ID NO: 64 - protein, 1480 aa, Artificial Sequence
  SYNTHESIZED
MDKKYSIGLDIGTNSVGWAVITDEYKVPSKKFKVLGNTDRHSIKKNLIGALLFDSGETAEATRLKRTARRRYTRRKNRICYLQEIFSNEMAKVDDSFFHRLEESFLVEEDKKHERHPIFGNIVDEVAYHEKYPTIYHLRKKLVDSTDKADLRLIYLALAHMIKFRGHFLIEGDLNPDNSDVDKLFIQLVQTYNQLFEENPINASGVDAKAILSARLSKSRRLENLIAQLPGEKKNGLFGNLIALSLGLTPNFKSNFDLAEDAKLQLSKDTYDDDLDNLLAQIGDQYADLFLAAKNLSDAILLSDILRVNTEITKAPLSASMIKRYDEHHQDLTLLKALVRQQLPEKYKEIFFDQSKNGYAGYIDGGASQEEFYKFIKPILEKMDGTEELLVKLNREDLLRKQRTFDNGSIPHQIHLGELHAILRRQEDFYPFLKDNREKIEKILTFRIPYYVGPLARGNSRFAWMTRKSEETITPWNFEEVVDKGASAQSFIERMTNFDKNLPNEKVLPKHSLLYEYFTVYNELTKVKYVTEGMRKPAFLSGEQKKAIVDLLFKTNRKVTVKQLKEDYFKKIECFDSVEISGVEDRFNASLGTYHDLLKIIKDKDFLDNEENEDILEDIVLTLTLFEDREMIEERLKTYAHLFDDKVMKQLKRRRYTGWGRLSRKLINGIRDKQSGKTILDFLKSDGFANRNFMQLIHDDSLTFKEDIQKAQVSGQGDSLHEHIANLAGSPAIKKGILQTVKIVDELVKVMGHKPENIVIEMARENQTTQKGQKNSRERMKRIEEGIKELGSQILKEHPVENTQLQNEKLYLYYLQNGRDMYVDQELDINRLSDYDVDHIVPQSFIKDDSIDNKVLTRSDKNRGKSDNVPSEEVVKKMKNYWRQLLNAKLITQRKFDNLTKAERGGLSELDKAGFIKRQLVETRQITKHVAQILDSRMNTKYDENDKLIREVKVITLKSKLVSDFRKDFQFYKVREINNYHHAHDAYLNAVVGTALIKKYPKLESEFVYGDYKVYDVRKMIAKSEQEIGKATAKYFFYSNIMNFFKTEITLANGEIRKRPLIETNGETGEIVWDKGRDFATVRKVLSMPQVNIVKKTEVQTGGFSKESILPKRNSDKLIARKKDWDPKKYGGFDSPTVAYSVLVVAKVEKGKSKKLKSVKELLGITIMERSSFEKNPIDFLEAKGYKEVKKDLIIKLPKYSLFELENGRKRMLASAGELQKGNELALPSKYVNFLYLASHYEKLKGSPEDNEQKQLFVEQHKHYLDEIIEQISEFSKRVILADANLDKVLSAYNKHRDKPIREQAENIIHLFTLTNLGAPAAFKYFDTTIDRKRYTSTKEVLDATLIHQSITGLYETRIDLSQLGGDPKKKRKVLEGGGGSMPKRKSPENTEGKDGSKVTKQEPTRRSARLSAKPAPPKPEPKPRKTSAKKEPGAKISRGAKGKKEEKQEAGKEGTAPSENGETKAEEAQKTESVDNEGE

SEQ ID NO: 65 - protein, 1458 aa, Artificial Sequence
  SYNTHESIZED
MDKKYSIGLDIGTNSVGWAVITDEYKVPSKKFKVLGNTDRHSIKKNLIGALLFDSGETAEATRLKRTARRRYTRRKNRICYLQEIFSNEMAKVDDSFFHRLEESFLVEEDKKHERHPIFGNIVDEVAYHEKYPTIYHLRKKLVDSTDKADLRLIYLALAHMIKFRGHFLIEGDLNPDNSDVDKLFIQLVQTYNQLFEENPINASGVDAKAILSARLSKSRRLENLIAQLPGEKKNGLFGNLIALSLGLTPNFKSNFDLAEDAKLQLSKDTYDDDLDNLLAQIGDQYADLFLAAKNLSDAILLSDILRVNTEITKAPLSASMIKRYDEHHQDLTLLKALVRQQLPEKYKEIFFDQSKNGYAGYIDGGASQEEFYKFIKPILEKMDGTEELLVKLNREDLLRKQRTFDNGSIPHQIHLGELHAILRRQEDFYPFLKDNREKIEKILTFRIPYYVGPLARGNSRFAWMTRKSEETITPWNFEEVVDKGASAQSFIERMTNFDKNLPNEKVLPKHSLLYEYFTVYNELTKVKYVTEGMRKPAFLSGEQKKAIVDLLFKTNRKVTVKQLKEDYFKKIECFDSVEISGVEDRFNASLGTYHDLLKIIKDKDFLDNEENEDILEDIVLTLTLFEDREMIEERLKTYAHLFDDKVMKQLKRRRYTGWGRLSRKLINGIRDKQSGKTILDFLKSDGFANRNFMQLIHDDSLTFKEDIQKAQVSGQGDSLHEHIANLAGSPAIKKGILQTVKIVDELVKVMGHKPENIVIEMARENQTTQKGQKNSRERMKRIEEGIKELGSQILKEHPVENTQLQNEKLYLYYLQNGRDMYVDQELDINRLSDYDVDHIVPQSFIKDDSIDNKVLTRSDKNRGKSDNVPSEEVVKKMKNYWRQLLNAKLITQRKFDNLTKAERGGLSELDKAGFIKRQLVETRQITKHVAQILDSRMNTKYDENDKLIREVKVITLKSKLVSDFRKDFQFYKVREINNYHHAHDAYLNAVVGTALIKKYPKLESEFVYGDYKVYDVRKMIAKSEQEIGKATAKYFFYSNIMNFFKTEITLANGEIRKRPLIETNGETGEIVWDKGRDFATVRKVLSMPQVNIVKKTEVQTGGFSKESILPKRNSDKLIARKKDWDPKKYGGFDSPTVAYSVLVVAKVEKGKSKKLKSVKELLGITIMERSSFEKNPIDFLEAKGYKEVKKDLIIKLPKYSLFELENGRKRMLASAGELQKGNELALPSKYVNFLYLASHYEKLKGSPEDNEQKQLFVEQHKHYLDEIIEQISEFSKRVILADANLDKVLSAYNKHRDKPIREQAENIIHLFTLTNLGAPAAFKYFDTTIDRKRYTSTKEVLDATLIHQSITGLYETRIDLSQLGGDPKKKRKVLEGGGGSMPKRKSPENTEGKDGSKVTKQEPTRRSARLSAKPAPPKPEPKPRKTSAKKEPGAKISRGAKGKKEEKQEAGKEGTEN

SEQ ID NO: 66 - protein, 1461 aa, Artificial Sequence
  SYNTHESIZED
MDKKYSIGLDIGTNSVGWAVITDEYKVPSKKFKVLGNTDRHSIKKNLIGALLFDSGETAEATRLKRTARRRYTRRKNRICYLQEIFSNEMAKVDDSFFHRLEESFLVEEDKKHERHPIFGNIVDEVAYHEKYPTIYHLRKKLVDSTDKADLRLIYLALAHMIKFRGHFLIEGDLNPDNSDVDKLFIQLVQTYNQLFEENPINASGVDAKAILSARLSKSRRLENLIAQLPGEKKNGLFGNLIALSLGLTPNFKSNFDLAEDAKLQLSKDTYDDDLDNLLAQIGDQYADLFLAAKNLSDAILLSDILRVNTEITKAPLSASMIKRYDEHHQDLTLLKALVRQQLPEKYKEIFFDQSKNGYAGYIDGGASQEEFYKFIKPILEKMDGTEELLVKLNREDLLRKQRTFDNGSIPHQIHLGELHAILRRQEDFYPFLKDNREKIEKILTFRIPYYVGPLARGNSRFAWMTRKSEETITPWNFEEVVDKGASAQSFIERMTNFDKNLPNEKVLPKHSLLYEYFTVYNELTKVKYVTEGMRKPAFLSGEQKKAIVDLLFKTNRKVTVKQLKEDYFKKIECFDSVEISGVEDRFNASLGTYHDLLKIIKDKDFLDNEENEDILEDIVLTLTLFEDREMIEERLKTYAHLFDDKVMKQLKRRRYTGWGRLSRKLINGIRDKQSGKTILDFLKSDGFANRNFMQLIHDDSLTFKEDIQKAQVSGQGDSLHEHIANLAGSPAIKKGILQTVKIVDELVKVMGHKPENIVIEMARENQTTQKGQKNSRERMKRIEEGIKELGSQILKEHPVENTQLQNEKLYLYYLQNGRDMYVDQELDINRLSDYDVDHIVPQSFIKDDSIDNKVLTRSDKNRGKSDNVPSEEVVKKMKNYWRQLLNAKLITQRKFDNLTKAERGGLSELDKAGFIKRQLVETRQITKHVAQILDSRMNTKYDENDKLIREVKVITLKSKLVSDFRKDFQFYKVREINNYHHAHDAYLNAVVGTALIKKYPKLESEFVYGDYKVYDVRKMIAKSEQEIGKATAKYFFYSNIMNFFKTEITLANGEIRKRPLIETNGETGEIVWDKGRDFATVRKVLSMPQVNIVKKTEVQTGGFSKESILPKRNSDKLIARKKDWDPKKYGGFDSPTVAYSVLVVAKVEKGKSKKLKSVKELLGITIMERSSFEKNPIDFLEAKGYKEVKKDLIIKLPKYSLFELENGRKRMLASAGELQKGNELALPSKYVNFLYLASHYEKLKGSPEDNEQKQLFVEQHKHYLDEIIEQISEFSKRVILADANLDKVLSAYNKHRDKPIREQAENIIHLFTLTNLGAPAAFKYFDTTIDRKRYTSTKEVLDATLIHQSITGLYETRIDLSQLGGDPKKKRKVLEGGGGSSTDHPKYSDMIVAAIQAEKNRAGSSRQSIQKYIKSHYKVGENADSQIKLSIKRLVTTGVLKQTKGVGASGSFRLAKSDEP

SEQ ID NO: 67 - protein, 1745 aa, Artificial Sequence
  SYNTHESIZED
LLNPTKRERKENYSIDNYYKDVLNTGRSSTPSHPRMPKPHVFHSHQLQPPQLKVLYEKERMWTAKKTGYVPTMDDVKAAYGDISDEEEKKQKLELLKLSVNNSQPLTEEEEKMKADWESEGFTNWNKLEFRKFITVSGKYGRNSIQAIARELAPGKTLEEVRAYAKAFWSNIERIEDYEKYLKIIENEEEKIKRVKMQQEALRRKLSEYKNPFFDLKLKHPPSSNNKRTYSEEEDRFILLMLFKYGLDRDDVYELVRDEIRDCPLFELDFYFRSRTPVELARRGNTLLQCLEKEFNAGIVLDDATKDRMKKEDENGKRIREEFADQTANEKENVDGVESKKAKIEDTSNVGTEQLVAEKIPENETTHTGSGMDKKYSIGLDIGTNSVGWAVITDEYKVPSKKFKVLGNTDRHSIKKNLIGALLFDSGETAEATRLKRTARRRYTRRKNRICYLQEIFSNEMAKVDDSFFHRLEESFLVEEDKKHERHPIFGNIVDEVAYHEKYPTIYHLRKKLVDSTDKADLRLIYLALAHMIKFRGHFLIEGDLNPDNSDVDKLFIQLVQTYNQLFEENPINASGVDAKAILSARLSKSRRLENLIAQLPGEKKNGLFGNLIALSLGLTPNFKSNFDLAEDAKLQLSKDTYDDDLDNLLAQIGDQYADLFLAAKNLSDAILLSDILRVNTEITKAPLSASMIKRYDEHHQDLTLLKALVRQQLPEKYKEIFFDQSKNGYAGYIDGGASQEEFYKFIKPILEKMDGTEELLVKLNREDLLRKQRTFDNGSIPHQIHLGELHAILRRQEDFYPFLKDNREKIEKILTFRIPYYVGPLARGNSRFAWMTRKSEETITPWNFEEVVDKGASAQSFIERMTNFDKNLPNEKVLPKHSLLYEYFTVYNELTKVKYVTEGMRKPAFLSGEQKKAIVDLLFKTNRKVTVKQLKEDYFKKIECFDSVEISGVEDRFNASLGTYHDLLKIIKDKDFLDNEENEDILEDIVLTLTLFEDREMIEERLKTYAHLFDDKVMKQLKRRRYTGWGRLSRKLINGIRDKQSGKTILDFLKSDGFANRNFMQLIHDDSLTFKEDIQKAQVSGQGDSLHEHIANLAGSPAIKKGILQTVKIVDELVKVMGHKPENIVIEMARENQTTQKGQKNSRERMKRIEEGIKELGSQILKEHPVENTQLQNEKLYLYYLQNGRDMYVDQELDINRLSDYDVDHIVPQSFIKDDSIDNKVLTRSDKNRGKSDNVPSEEVVKKMKNYWRQLLNAKLITQRKFDNLTKAERGGLSELDKAGFIKRQLVETRQITKHVAQILDSRMNTKYDENDKLIREVKVITLKSKLVSDFRKDFQFYKVREINNYHHAHDAYLNAVVGTALIKKYPKLESEFVYGDYKVYDVRKMIAKSEQEIGKATAKYFFYSNIMNFFKTEITLANGEIRKRPLIETNGETGEIVWDKGRDFATVRKVLSMPQVNIVKKTEVQTGGFSKESILPKRNSDKLIARKKDWDPKKYGGFDSPTVAYSVLVVAKVEKGKSKKLKSVKELLGITIMERSSFEKNPIDFLEAKGYKEVKKDLIIKLPKYSLFELENGRKRMLASAGELQKGNELALPSKYVNFLYLASHYEKLKGSPEDNEQKQLFVEQHKHYLDEIIEQISEFSKRVILADANLDKVLSAYNKHRDKPIREQAENIIHLFTLTNLGAPAAFKYFDTTIDRKRYTSTKEVLDATLIHQSITGLYETRIDLSQLGGDPKKKRKV

SEQ ID NO: 68 - protein, 1650 aa, Artificial Sequence
  SYNTHESIZED
MDKKYSIGLDIGTNSVGWAVITDEYKVPSKKFKVLGNTDRHSIKKNLIGALLFDSGETAEATRLKRTARRRYTRRKNRICYLQEIFSNEMAKVDDSFFHRLEESFLVEEDKKHERHPIFGNIVDEVAYHEKYPTIYHLRKKLVDSTDKADLRLIYLALAHMIKFRGHFLIEGDLNPDNSDVDKLFIQLVQTYNQLFEENPINASGVDAKAILSARLSKSRRLENLIAQLPGEKKNGLFGNLIALSLGLTPNFKSNFDLAEDAKLQLSKDTYDDDLDNLLAQIGDQYADLFLAAKNLSDAILLSDILRVNTEITKAPLSASMIKRYDEHHQDLTLLKALVRQQLPEKYKEIFFDQSKNGYAGYIDGGASQEEFYKFIKPILEKMDGTEELLVKLNREDLLRKQRTFDNGSIPHQIHLGELHAILRRQEDFYPFLKDNREKIEKILTFRIPYYVGPLARGNSRFAWMTRKSEETITPWNFEEVVDKGASAQSFIERMTNFDKNLPNEKVLPKHSLLYEYFTVYNELTKVKYVTEGMRKPAFLSGEQKKAIVDLLFKTNRKVTVKQLKEDYFKKIECFDSVEISGVEDRFNASLGTYHDLLKIIKDKDFLDNEENEDILEDIVLTLTLFEDREMIEERLKTYAHLFDDKVMKQLKRRRYTGWGRLSRKLINGIRDKQSGKTILDFLKSDGFANRNFMQLIHDDSLTFKEDIQKAQVSGQGDSLHEHIANLAGSPAIKKGILQTVKIVDELVKVMGHKPENIVIEMARENQTTQKGQKNSRERMKRIEEGIKELGSQILKEHPVENTQLQNEKLYLYYLQNGRDMYVDQELDINRLSDYDVDHIVPQSFIKDDSIDNKVLTRSDKNRGKSDNVPSEEVVKKMKNYWRQLLNAKLITQRKFDNLTKAERGGLSELDKAGFIKRQLVETRQITKHVAQILDSRMNTKYDENDKLIREVKVITLKSKLVSDFRKDFQFYKVREINNYHHAHDAYLNAVVGTALIKKYPKLESEFVYGDYKVYDVRKMIAKSEQEIGKATAKYFFYSNIMNFFKTEITLANGEIRKRPLIETNGETGEIVWDKGRDFATVRKVLSMPQVNIVKKTEVQTGGFSKESILPKRNSDKLIARKKDWDPKKYGGFDSPTVAYSVLVVAKVEKGKSKKLKSVKELLGITIMERSSFEKNPIDFLEAKGYKEVKKDLIIKLPKYSLFELENGRKRMLASAGELQKGNELALPSKYVNFLYLASHYEKLKGSPEDNEQKQLFVEQHKHYLDEIIEQISEFSKRVILADANLDKVLSAYNKHRDKPIREQAENIIHLFTLTNLGAPAAFKYFDTTIDRKRYTSTKEVLDATLIHQSITGLYETRIDLSQLGGDPKKKRKVLEGGGGSDMDSIGESEVRALYKAILKFGNLKEILDELIADGTLPVKSFEKYGETYDEMMEAAKDCVHEEEKNRKEILEKLEKHATAYRAKLKSGEIKAENQPKDNPLTRLSLKKREKKAVLFNFKGVKSLNAESLLSRVEDLKYLKNLINSNYKDDPLKFSLGNNTPKPVQNWSSNWTKEEDEKLLIGVFKYGYGSWTQIRDDPFLGITDKIFLNEVHNPVAKKSASSSDTTPTPSKKGKGITGSSKKVPGAIHLGRRVDYLLSFLRGGLNTKSPS

SEQ ID NO: 69 - protein, 1568 aa, Artificial Sequence
  SYNTHESIZED
MPKRKVSSAEGAAKEEPKRRSARLSAKPPAKVEAKPKKAAAKDKSSDKKVQTKGKRGAKGKQAEVANQETKEDLPAENGETKTEESPASDEAGEKEAKSDTGSGMDKKYSIGLDIGTNSVGWAVITDEYKVPSKKFKVLGNTDRHSIKKNLIGALLFDSGETAEATRLKRTARRRYTRRKNRICYLQEIFSNEMAKVDDSFFHRLEESFLVEEDKKHERHPIFGNIVDEVAYHEKYPTIYHLRKKLVDSTDKADLRLIYLALAHMIKFRGHFLIEGDLNPDNSDVDKLFIQLVQTYNQLFEENPINASGVDAKAILSARLSKSRRLENLIAQLPGEKKNGLFGNLIALSLGLTPNFKSNFDLAEDAKLQLSKDTYDDDLDNLLAQIGDQYADLFLAAKNLSDAILLSDILRVNTEITKAPLSASMIKRYDEHHQDLTLLKALVRQQLPEKYKEIFFDQSKNGYAGYIDGGASQEEFYKFIKPILEKMDGTEELLVKLNREDLLRKQRTFDNGSIPHQIHLGELHAILRRQEDFYPFLKDNREKIEKILTFRIPYYVGPLARGNSRFAWMTRKSEETITPWNFEEVVDKGASAQSFIERMTNFDKNLPNEKVLPKHSLLYEYFTVYNELTKVKYVTEGMRKPAFLSGEQKKAIVDLLFKTNRKVTVKQLKEDYFKKIECFDSVEISGVEDRFNASLGTYHDLLKIIKDKDFLDNEENEDILEDIVLTLTLFEDREMIEERLKTYAHLFDDKVMKQLKRRRYTGWGRLSRKLINGIRDKQSGKTILDFLKSDGFANRNFMQLIHDDSLTFKEDIQKAQVSGQGDSLHEHIANLAGSPAIKKGILQTVKIVDELVKVMGHKPENIVIEMARENQTTQKGQKNSRERMKRIEEGIKELGSQILKEHPVENTQLQNEKLYLYYLQNGRDMYVDQELDINRLSDYDVDHIVPQSFIKDDSIDNKVLTRSDKNRGKSDNVPSEEVVKKMKNYWRQLLNAKLITQRKFDNLTKAERGGLSELDKAGFIKRQLVETRQITKHVAQILDSRMNTKYDENDKLIREVKVITLKSKLVSDFRKDFQFYKVREINNYHHAHDAYLNAVVGTALIKKYPKLESEFVYGDYKVYDVRKMIAKSEQEIGKATAKYFFYSNIMNFFKTEITLANGEIRKRPLIETNGETGEIVWDKGRDFATVRKVLSMPQVNIVKKTEVQTGGFSKESILPKRNSDKLIARKKDWDPKKYGGFDSPTVAYSVLVVAKVEKGKSKKLKSVKELLGITIMERSSFEKNPIDFLEAKGYKEVKKDLIIKLPKYSLFELENGRKRMLASAGELQKGNELALPSKYVNFLYLASHYEKLKGSPEDNEQKQLFVEQHKHYLDEIIEQISEFSKRVILADANLDKVLSAYNKHRDKPIREQAENIIHLFTLTNLGAPAAFKYFDTTIDRKRYTSTKEVLDATLIHQSITGLYETRIDLSQLGGDPKKKRKVLEGGGGSGKGDPKKPRGKMSSYAFFVQTCREEHKKKHPDASVNFSEFSKKCSERWKTMSAKEKGKFEDMAKADKARYEREMKTYIPPKGE

SEQ ID NO: 70 - protein, 1565 aa, Artificial Sequence
  SYNTHESIZED
MPKRKVSSAEGAAKEEPKRRSARLSAKPPAKVEAKPKKAAAKDKSSDKKVQTKGKRGAKGKQAEVANQETKEDLPAENGETKTEESPASDEAGEKEAKSDTGSGMDKKYSIGLDIGTNSVGWAVITDEYKVPSKKFKVLGNTDRHSIKKNLIGALLFDSGETAEATRLKRTARRRYTRRKNRICYLQEIFSNEMAKVDDSFFHRLEESFLVEEDKKHERHPIFGNIVDEVAYHEKYPTIYHLRKKLVDSTDKADLRLIYLALAHMIKFRGHFLIEGDLNPDNSDVDKLFIQLVQTYNQLFEENPINASGVDAKAILSARLSKSRRLENLIAQLPGEKKNGLFGNLIALSLGLTPNFKSNFDLAEDAKLQLSKDTYDDDLDNLLAQIGDQYADLFLAAKNLSDAILLSDILRVNTEITKAPLSASMIKRYDEHHQDLTLLKALVRQQLPEKYKEIFFDQSKNGYAGYIDGGASQEEFYKFIKPILEKMDGTEELLVKLNREDLLRKQRTFDNGSIPHQIHLGELHAILRRQEDFYPFLKDNREKIEKILTFRIPYYVGPLARGNSRFAWMTRKSEETITPWNFEEVVDKGASAQSFIERMTNFDKNLPNEKVLPKHSLLYEYFTVYNELTKVKYVTEGMRKPAFLSGEQKKAIVDLLFKTNRKVTVKQLKEDYFKKIECFDSVEISGVEDRFNASLGTYHDLLKIIKDKDFLDNEENEDILEDIVLTLTLFEDREMIEERLKTYAHLFDDKVMKQLKRRRYTGWGRLSRKLINGIRDKQSGKTILDFLKSDGFANRNFMQLIHDDSLTFKEDIQKAQVSGQGDSLHEHIANLAGSPAIKKGILQTVKIVDELVKVMGHKPENIVIEMARENQTTQKGQKNSRERMKRIEEGIKELGSQILKEHPVENTQLQNEKLYLYYLQNGRDMYVDQELDINRLSDYDVDHIVPQSFIKDDSIDNKVLTRSDKNRGKSDNVPSEEVVKKMKNYWRQLLNAKLITQRKFDNLTKAERGGLSELDKAGFIKRQLVETRQITKHVAQILDSRMNTKYDENDKLIREVKVITLKSKLVSDFRKDFQFYKVREINNYHHAHDAYLNAVVGTALIKKYPKLESEFVYGDYKVYDVRKMIAKSEQEIGKATAKYFFYSNIMNFFKTEITLANGEIRKRPLIETNGETGEIVWDKGRDFATVRKVLSMPQVNIVKKTEVQTGGFSKESILPKRNSDKLIARKKDWDPKKYGGFDSPTVAYSVLVVAKVEKGKSKKLKSVKELLGITIMERSSFEKNPIDFLEAKGYKEVKKDLIIKLPKYSLFELENGRKRMLASAGELQKGNELALPSKYVNFLYLASHYEKLKGSPEDNEQKQLFVEQHKHYLDEIIEQISEFSKRVILADANLDKVLSAYNKHRDKPIREQAENIIHLFTLTNLGAPAAFKYFDTTIDRKRYTSTKEVLDATLIHQSITGLYETRIDLSQLGGDPKKKRKVLEGGGGSSTDHPKYSDMIVAAIQAEKNRAGSSRQSIQKYIKSHYKVGENADSQIKLSIKRLVTTGVLKQTKGVGASGSFRLAKSDEP

SEQ ID NO: 71 - protein, 1754 aa, Artificial Sequence
  SYNTHESIZED
MPKRKVSSAEGAAKEEPKRRSARLSAKPPAKVEAKPKKAAAKDKSSDKKVQTKGKRGAKGKQAEVANQETKEDLPAENGETKTEESPASDEAGEKEAKSDTGSGMDKKYSIGLDIGTNSVGWAVITDEYKVPSKKFKVLGNTDRHSIKKNLIGALLFDSGETAEATRLKRTARRRYTRRKNRICYLQEIFSNEMAKVDDSFFHRLEESFLVEEDKKHERHPIFGNIVDEVAYHEKYPTIYHLRKKLVDSTDKADLRLIYLALAHMIKFRGHFLIEGDLNPDNSDVDKLFIQLVQTYNQLFEENPINASGVDAKAILSARLSKSRRLENLIAQLPGEKKNGLFGNLIALSLGLTPNFKSNFDLAEDAKLQLSKDTYDDDLDNLLAQIGDQYADLFLAAKNLSDAILLSDILRVNTEITKAPLSASMIKRYDEHHQDLTLLKALVRQQLPEKYKEIFFDQSKNGYAGYIDGGASQEEFYKFIKPILEKMDGTEELLVKLNREDLLRKQRTFDNGSIPHQIHLGELHAILRRQEDFYPFLKDNREKIEKILTFRIPYYVGPLARGNSRFAWMTRKSEETITPWNFEEVVDKGASAQSFIERMTNFDKNLPNEKVLPKHSLLYEYFTVYNELTKVKYVTEGMRKPAFLSGEQKKAIVDLLFKTNRKVTVKQLKEDYFKKIECFDSVEISGVEDRFNASLGTYHDLLKIIKDKDFLDNEENEDILEDIVLTLTLFEDREMIEERLKTYAHLFDDKVMKQLKRRRYTGWGRLSRKLINGIRDKQSGKTILDFLKSDGFANRNFMQLIHDDSLTFKEDIQKAQVSGQGDSLHEHIANLAGSPAIKKGILQTVKIVDELVKVMGHKPENIVIEMARENQTTQKGQKNSRERMKRIEEGIKELGSQILKEHPVENTQLQNEKLYLYYLQNGRDMYVDQELDINRLSDYDVDHIVPQSFIKDDSIDNKVLTRSDKNRGKSDNVPSEEVVKKMKNYWRQLLNAKLITQRKFDNLTKAERGGLSELDKAGFIKRQLVETRQITKHVAQILDSRMNTKYDENDKLIREVKVITLKSKLVSDFRKDFQFYKVREINNYHHAHDAYLNAVVGTALIKKYPKLESEFVYGDYKVYDVRKMIAKSEQEIGKATAKYFFYSNIMNFFKTEITLANGEIRKRPLIETNGETGEIVWDKGRDFATVRKVLSMPQVNIVKKTEVQTGGFSKESILPKRNSDKLIARKKDWDPKKYGGFDSPTVAYSVLVVAKVEKGKSKKLKSVKELLGITIMERSSFEKNPIDFLEAKGYKEVKKDLIIKLPKYSLFELENGRKRMLASAGELQKGNELALPSKYVNFLYLASHYEKLKGSPEDNEQKQLFVEQHKHYLDEIIEQISEFSKRVILADANLDKVLSAYNKHRDKPIREQAENIIHLFTLTNLGAPAAFKYFDTTIDRKRYTSTKEVLDATLIHQSITGLYETRIDLSQLGGDPKKKRKVLEGGGGSDMDSIGESEVRALYKAILKFGNLKEILDELIADGTLPVKSFEKYGETYDEMMEAAKDCVHEEEKNRKEILEKLEKHATAYRAKLKSGEIKAENQPKDNPLTRLSLKKREKKAVLFNFKGVKSLNAESLLSRVEDLKYLKNLINSNYKDDPLKFSLGNNTPKPVQNWSSNWTKEEDEKLLIGVFKYGYGSWTQIRDDPFLGITDKIFLNEVHNPVAKKSASSSDTTPTPSKKGKGITGSSKKVPGAIHLGRRVDYLLSFLRGGLNTKSPS

SEQ ID NO: 72 - protein, 1331 aa, Artificial Sequence
  SYNTHESIZED
MPKRKVSSAEGAAKEEPKRRSARLSAKPPAKVEAKPKKAAAKDKSSDKKVQTKGKRGAKGKQAEVANQETKEDLPAENGETKTEESPASDEAGEKEAKSDTGSGMTNGKILGLDIGIASVGVGIIEAKTGKVVHANSRLFSAANAENNAERRGFRGSRRLNRRKKHRVKRVRDLFEKYGIVTDFRNLNLNPYELRVKGLTEQLKNEELFAALRTISKRRGISYLDDAEDDSTGSTDYAKSIDENRRLLKNKTPGQIQLERLEKYGQLRGNFTVYDENGEAHRLINVFSTSDYEKEARKILETQADYNKKITAEFIDDYVEILTQKRKYYHGPGNEKSRTDYGRFRTDGTTLENIFGILIGKCNFYPDEYRASKASYTAQEYNFLNDLNNLKVSTETGKLSTEQKESLVEFAKNTATLGPAKLLKEIAKILDCKVDEIKGYREDDKGKPDLHTFEPYRKLKFNLESINIDDLSREVIDKLADILTLNTEREGIEDAIKRNLPNQFTEEQISEIIKVRKSQSTAFNKGWHSFSAKLMNELIPELYATSDEQMTILTRLEKFKVNKKSSKNTKTIDEKEVTDEIYNPVVAKSVRQTIKIINAAVKKYGDFDKIVIEMPRDKNADDEKKFIDKRNKENKKEKDDALKRAAYLYNSSDKLPDEVFHGNKQLETKIRLWYQQGERCLYSGKPISIQELVHNSNNFEIDHILPLSLSFDDSLANKVLVYAWTNQEKGQKTPYQVIDSMDAAWSFREMKDYVLKQKGLGKKKRDYLLTTENIDKIEVKKKFIERNLVDTRYASRVVLNSLQSALRELGKDTKVSVVRGQFTSQLRRKWKIDKSRETYHHHAVDALIIAASSQLKLWEKQDNPMFVDYGKNQVVDKQTGEILSVSDDEYKELVFQPPYQGFVNTISSKGFEDEILFSYQVDSKYNRKVSDATIYSTRKAKIGKDKKEETYVLGKIKDIYSQNGFDTFIKKYNKDKTQFLMYQKDSLTWENVIEVILRDYPTTKKSEDGKNDVKCNPFEEYRRENGLICKYSKKGKGTPIKSLKYYDKKLGNCIDITPEESRNKVILQSINPWRADVYFNPETLKYELMGLKYSDLSFEKGTGNYHISQEKYDAIKEKEGIGKKSEFKFTLYRNDLILIKDIASGEQEIYRFLSRTMPNVNHYVELKPYDKEKFDNVQELVEALGEADKVGRCIKGLNKPNISIYKVRTDVLGNKYFVKKKGDKPKLDFKNNKKPKKKRKVLEGGGGSGKGDPKKPRGKMSSYAFFVQTCREEHKKKHPDASVNFSEFSKKCSERWKTMSAKEKGKFEDMAKADKARYEREMKTYIPPKGE

SEQ ID NO: 73 - protein, 1328 aa, Artificial Sequence
  SYNTHESIZED
MPKRKVSSAEGAAKEEPKRRSARLSAKPPAKVEAKPKKAAAKDKSSDKKVQTKGKRGAKGKQAEVANQETKEDLPAENGETKTEESPASDEAGEKEAKSDTGSGMTNGKILGLDIGIASVGVGIIEAKTGKVVHANSRLFSAANAENNAERRGFRGSRRLNRRKKHRVKRVRDLFEKYGIVTDFRNLNLNPYELRVKGLTEQLKNEELFAALRTISKRRGISYLDDAEDDSTGSTDYAKSIDENRRLLKNKTPGQIQLERLEKYGQLRGNFTVYDENGEAHRLINVFSTSDYEKEARKILETQADYNKKITAEFIDDYVEILTQKRKYYHGPGNEKSRTDYGRFRTDGTTLENIFGILIGKCNFYPDEYRASKASYTAQEYNFLNDLNNLKVSTETGKLSTEQKESLVEFAKNTATLGPAKLLKEIAKILDCKVDEIKGYREDDKGKPDLHTFEPYRKLKFNLESINIDDLSREVIDKLADILTLNTEREGIEDAIKRNLPNQFTEEQISEIIKVRKSQSTAFNKGWHSFSAKLMNELIPELYATSDEQMTILTRLEKFKVNKKSSKNTKTIDEKEVTDEIYNPVVAKSVRQTIKIINAAVKKYGDFDKIVIEMPRDKNADDEKKFIDKRNKENKKEKDDALKRAAYLYNSSDKLPDEVFHGNKQLETKIRLWYQQGERCLYSGKPISIQELVHNSNNFEIDHILPLSLSFDDSLANKVLVYAWTNQEKGQKTPYQVIDSMDAAWSFREMKDYVLKQKGLGKKKRDYLLTTENIDKIEVKKKFIERNLVDTRYASRVVLNSLQSALRELGKDTKVSVVRGQFTSQLRRKWKIDKSRETYHHHAVDALIIAASSQLKLWEKQDNPMFVDYGKNQVVDKQTGEILSVSDDEYKELVFQPPYQGFVNTISSKGFEDEILFSYQVDSKYNRKVSDATIYSTRKAKIGKDKKEETYVLGKIKDIYSQNGFDTFIKKYNKDKTQFLMYQKDSLTWENVIEVILRDYPTTKKSEDGKNDVKCNPFEEYRRENGLICKYSKKGKGTPIKSLKYYDKKLGNCIDITPEESRNKVILQSINPWRADVYFNPETLKYELMGLKYSDLSFEKGTGNYHISQEKYDAIKEKEGIGKKSEFKFTLYRNDLILIKDIASGEQEIYRFLSRTMPNVNHYVELKPYDKEKFDNVQELVEALGEADKVGRCIKGLNKPNISIYKVRTDVLGNKYFVKKKGDKPKLDFKNNKKPKKKRKVLEGGGGSSTDHPKYSDMIVAAIQAEKNRAGSSRQSIQKYIKSHYKVGENADSQIKLSIKRLVTTGVLKQTKGVGASGSFRLAKSDEP

SEQ ID NO: 74 - protein, 1517 aa, Artificial Sequence
  SYNTHESIZED
MPKRKVSSAEGAAKEEPKRRSARLSAKPPAKVEAKPKKAAAKDKSSDKKVQTKGKRGAKGKQAEVANQETKEDLPAENGETKTEESPASDEAGEKEAKSDTGSGMTNGKILGLDIGIASVGVGIIEAKTGKVVHANSRLFSAANAENNAERRGFRGSRRLNRRKKHRVKRVRDLFEKYGIVTDFRNLNLNPYELRVKGLTEQLKNEELFAALRTISKRRGISYLDDAEDDSTGSTDYAKSIDENRRLLKNKTPGQIQLERLEKYGQLRGNFTVYDENGEAHRLINVFSTSDYEKEARKILETQADYNKKITAEFIDDYVEILTQKRKYYHGPGNEKSRTDYGRFRTDGTTLENIFGILIGKCNFYPDEYRASKASYTAQEYNFLNDLNNLKVSTETGKLSTEQKESLVEFAKNTATLGPAKLLKEIAKILDCKVDEIKGYREDDKGKPDLHTFEPYRKLKFNLESINIDDLSREVIDKLADILTLNTEREGIEDAIKRNLPNQFTEEQISEIIKVRKSQSTAFNKGWHSFSAKLMNELIPELYATSDEQMTILTRLEKFKVNKKSSKNTKTIDEKEVTDEIYNPVVAKSVRQTIKIINAAVKKYGDFDKIVIEMPRDKNADDEKKFIDKRNKENKKEKDDALKRAAYLYNSSDKLPDEVFHGNKQLETKIRLWYQQGERCLYSGKPISIQELVHNSNNFEIDHILPLSLSFDDSLANKVLVYAWTNQEKGQKTPYQVIDSMDAAWSFREMKDYVLKQKGLGKKKRDYLLTTENIDKIEVKKKFIERNLVDTRYASRVVLNSLQSALRELGKDTKVSVVRGQFTSQLRRKWKIDKSRETYHHHAVDALIIAASSQLKLWEKQDNPMFVDYGKNQVVDKQTGEILSVSDDEYKELVFQPPYQGFVNTISSKGFEDEILFSYQVDSKYNRKVSDATIYSTRKAKIGKDKKEETYVLGKIKDIYSQNGFDTFIKKYNKDKTQFLMYQKDSLTWENVIEVILRDYPTTKKSEDGKNDVKCNPFEEYRRENGLICKYSKKGKGTPIKSLKYYDKKLGNCIDITPEESRNKVILQSINPWRADVYFNPETLKYELMGLKYSDLSFEKGTGNYHISQEKYDAIKEKEGIGKKSEFKFTLYRNDLILIKDIASGEQEIYRFLSRTMPNVNHYVELKPYDKEKFDNVQELVEALGEADKVGRCIKGLNKPNISIYKVRTDVLGNKYFVKKKGDKPKLDFKNNKKPKKKRKVLEGGGGSDMDSIGESEVRALYKAILKFGNLKEILDELIADGTLPVKSFEKYGETYDEMMEAAKDCVHEEEKNRKEILEKLEKHATAYRAKLKSGEIKAENQPKDNPLTRLSLKKREKKAVLFNFKGVKSLNAESLLSRVEDLKYLKNLINSNYKDDPLKFSLGNNTPKPVQNWSSNWTKEEDEKLLIGVFKYGYGSWTQIRDDPFLGITDKIFLNEVHNPVAKKSASSSDTTPTPSKKGKGITGSSKKVPGAIHLGRRVDYLLSFLRGGLNTKSPS

SEQ ID NO: 75 - protein, 1501 aa, Artificial Sequence
  SYNTHESIZED
MPKRKVSSAEGAAKEEPKRRSARLSAKPPAKVEAKPKKAAAKDKSSDKKVQTKGKRGAKGKQAEVANQETKEDLPAENGETKTEESPASDEAGEKEAKSDTGSGMSIYQEFVNKYSLSKTLRFELIPQGKTLENIKARGLILDDEKRAKDYKKAKQIIDKYHQFFIEEILSSVCISEDLLQNYSDVYFKLKKSDDDNLQKDFKSAKDTIKKQISEYIKDSEKFKNLFNQNLIDAKKGQESDLILWLKQSKDNGIELFKANSDITDIDEALEIIKSFKGWTTYFKGFHENRKNVYSSNDIPTSIIYRIVDDNLPKFLENKAKYESLKDKAPEAINYEQIKKDLAEELTFDIDYKTSEVNQRVFSLDEVFEIANFNNYLNQSGITKFNTIIGGKFVNGENTKRKGINEYINLYSQQINDKTLKKYKMSVLFKQILSDTESKSFVIDKLEDDSDVVTTMQSFYEQIAAFKTVEEKSIKETLSLLFDDLKAQKLDLSKIYFKNDKSLTDLSQQVFDDYSVIGTAVLEYITQQIAPKNLDNPSKKEQELIAKKTEKAKYLSLETIKLALEEFNKHRDIDKQCRFEEILANFAAIPMIFDEIAQNKDNLAQISIKYQNQGKKDLLQASAEDDVKAIKDLLDQTNNLLHKLKIFHISQSEDKANILDKDEHFYLVFEECYFELANIVPLYNKIRNYITQKPYSDEKFKLNFENSTLANGWDKNKEPDNTAILFIKDDKYYLGVMNKKNNKIFDDKAIKENKGEGYKKIVYKLLPGANKMLPKVFFSAKSIKFYNPSEDILRIRNHSTHTKNGSPQKGYEKFEFNIEDCRKFIDFYKQSISKHPEWKDFGFRFSDTQRYNSIDEFYREVENQGYKLTFENISESYIDSVVNQGKLYLFQIYNKDFSAYSKGRPNLHTLYWKALFDERNLQDVVYKLNGEAELFYRKQSIPKKITHPAKEAIANKNKDNPKKESVFEYDLIKDKRFTEDKFFFHCPITINFKSSGANKFNDEINLLLKEKANDVHILSIDRGERHLAYYTLVDGKGNIIKQDTFNIIGNDRMKTNYHDKLAAIEKDRDSARKDWKKINNIKEMKEGYLSQVVHEIAKLVIEYNAIVVFEDLNFGFKRGRFKVEKQVYQKLEKMLIEKLNYLVFKDNEFDKTGGVLRAYQLTAPFETFKKMGKQTGIIYYVPAGFTSKICPVTGFVNQLYPKYESVSKSQEFFSKFDKICYNLDKGYFEFSFDYKNFGDKAAKGKWTIASFGSRLINFRNSDKNHNWDTREVYPTKELEKLLKDYSIEYGHGECIKAAICGESDKKFFAKLTSVLNTILQMRNSKTGTELDYLISPVADVNGNFFDSRQAPKNMPQDADANGAYHIGLKGLMLLGRIKNNQEGKKLNLVIKNEEYFEFVQNRNNPKKKRKVLEGGGGSGKGDPKKPRGKMSSYAFFVQTCREEHKKKHPDASVNFSEFSKKCSERWKTMSAKEKGKFEDMAKADKARYEREMKTYIPPKGE

SEQ ID NO: 76 - protein, 1498 aa, Artificial Sequence
  SYNTHESIZED
MPKRKVSSAEGAAKEEPKRRSARLSAKPPAKVEAKPKKAAAKDKSSDKKVQTKGKRGAKGKQAEVANQETKEDLPAENGETKTEESPASDEAGEKEAKSDTGSGMSIYQEFVNKYSLSKTLRFELIPQGKTLENIKARGLILDDEKRAKDYKKAKQIIDKYHQFFIEEILSSVCISEDLLQNYSDVYFKLKKSDDDNLQKDFKSAKDTIKKQISEYIKDSEKFKNLFNQNLIDAKKGQESDLILWLKQSKDNGIELFKANSDITDIDEALEIIKSFKGWTTYFKGFHENRKNVYSSNDIPTSIIYRIVDDNLPKFLENKAKYESLKDKAPEAINYEQIKKDLAEELTFDIDYKTSEVNQRVFSLDEVFEIANFNNYLNQSGITKFNTIIGGKFVNGENTKRKGINEYINLYSQQINDKTLKKYKMSVLFKQILSDTESKSFVIDKLEDDSDVVTTMQSFYEQIAAFKTVEEKSIKETLSLLFDDLKAQKLDLSKIYFKNDKSLTDLSQQVFDDYSVIGTAVLEYITQQIAPKNLDNPSKKEQELIAKKTEKAKYLSLETIKLALEEFNKHRDIDKQCRFEEILANFAAIPMIFDEIAQNKDNLAQISIKYQNQGKKDLLQASAEDDVKAIKDLLDQTNNLLHKLKIFHISQSEDKANILDKDEHFYLVFEECYFELANIVPLYNKIRNYITQKPYSDEKFKLNFENSTLANGWDKNKEPDNTAILFIKDDKYYLGVMNKKNNKIFDDKAIKENKGEGYKKIVYKLLPGANKMLPKVFFSAKSIKFYNPSEDILRIRNHSTHTKNGSPQKGYEKFEFNIEDCRKFIDFYKQSISKHPEWKDFGFRFSDTQRYNSIDEFYREVENQGYKLTFENISESYIDSVVNQGKLYLFQIYNKDFSAYSKGRPNLHTLYWKALFDERNLQDVVYKLNGEAELFYRKQSIPKKITHPAKEAIANKNKDNPKKESVFEYDLIKDKRFTEDKFFFHCPITINFKSSGANKFNDEINLLLKEKANDVHILSIDRGERHLAYYTLVDGKGNIIKQDTFNIIGNDRMKTNYHDKLAAIEKDRDSARKDWKKINNIKEMKEGYLSQVVHEIAKLVIEYNAIVVFEDLNFGFKRGRFKVEKQVYQKLEKMLIEKLNYLVFKDNEFDKTGGVLRAYQLTAPFETFKKMGKQTGIIYYVPAGFTSKICPVTGFVNQLYPKYESVSKSQEFFSKFDKICYNLDKGYFEFSFDYKNFGDKAAKGKWTIASFGSRLINFRNSDKNHNWDTREVYPTKELEKLLKDYSIEYGHGECIKAAICGESDKKFFAKLTSVLNTILQMRNSKTGTELDYLISPVADVNGNFFDSRQAPKNMPQDADANGAYHIGLKGLMLLGRIKNNQEGKKLNLVIKNEEYFEFVQNRNNPKKKRKVLEGGGGSSTDHPKYSDMIVAAIQAEKNRAGSSRQSIQKYIKSHYKVGENADSQIKLSIKRLVTTGVLKQTKGVGASGSFRLAKSDEP

SEQ ID NO: 77 - protein, 1687 aa, Artificial Sequence
  SYNTHESIZED
MPKRKVSSAEGAAKEEPKRRSARLSAKPPAKVEAKPKKAAAKDKSSDKKVQTKGKRGAKGKQAEVANQETKEDLPAENGETKTEESPASDEAGEKEAKSDTGSGMSIYQEFVNKYSLSKTLRFELIPQGKTLENIKARGLILDDEKRAKDYKKAKQIIDKYHQFFIEEILSSVCISEDLLQNYSDVYFKLKKSDDDNLQKDFKSAKDTIKKQISEYIKDSEKFKNLFNQNLIDAKKGQESDLILWLKQSKDNGIELFKANSDITDIDEALEIIKSFKGWTTYFKGFHENRKNVYSSNDIPTSIIYRIVDDNLPKFLENKAKYESLKDKAPEAINYEQIKKDLAEELTFDIDYKTSEVNQRVFSLDEVFEIANFNNYLNQSGITKFNTIIGGKFVNGENTKRKGINEYINLYSQQINDKTLKKYKMSVLFKQILSDTESKSFVIDKLEDDSDVVTTMQSFYEQIAAFKTVEEKSIKETLSLLFDDLKAQKLDLSKIYFKNDKSLTDLSQQVFDDYSVIGTAVLEYITQQIAPKNLDNPSKKEQELIAKKTEKAKYLSLETIKLALEEFNKHRDIDKQCRFEEILANFAAIPMIFDEIAQNKDNLAQISIKYQNQGKKDLLQASAEDDVKAIKDLLDQTNNLLHKLKIFHISQSEDKANILDKDEHFYLVFEECYFELANIVPLYNKIRNYITQKPYSDEKFKLNFENSTLANGWDKNKEPDNTAILFIKDDKYYLGVMNKKNNKIFDDKAIKENKGEGYKKIVYKLLPGANKMLPKVFFSAKSIKFYNPSEDILRIRNHSTHTKNGSPQKGYEKFEFNIEDCRKFIDFYKQSISKHPEWKDFGFRFSDTQRYNSIDEFYREVENQGYKLTFENISESYIDSVVNQGKLYLFQIYNKDFSAYSKGRPNLHTLYWKALFDERNLQDVVYKLNGEAELFYRKQSIPKKITHPAKEAIANKNKDNPKKESVFEYDLIKDKRFTEDKFFFHCPITINFKSSGANKFNDEINLLLKEKANDVHILSIDRGERHLAYYTLVDGKGNIIKQDTFNIIGNDRMKTNYHDKLAAIEKDRDSARKDWKKINNIKEMKEGYLSQVVHEIAKLVIEYNAIVVFEDLNFGFKRGRFKVEKQVYQKLEKMLIEKLNYLVFKDNEFDKTGGVLRAYQLTAPFETFKKMGKQTGIIYYVPAGFTSKICPVTGFVNQLYPKYESVSKSQEFFSKFDKICYNLDKGYFEFSFDYKNFGDKAAKGKWTIASFGSRLINFRNSDKNHNWDTREVYPTKELEKLLKDYSIEYGHGECIKAAICGESDKKFFAKLTSVLNTILQMRNSKTGTELDYLISPVADVNGNFFDSRQAPKNMPQDADANGAYHIGLKGLMLLGRIKNNQEGKKLNLVIKNEEYFEFVQNRNNPKKKRKVLEGGGGSDMDSIGESEVRALYKAILKFGNLKEILDELIADGTLPVKSFEKYGETYDEMMEAAKDCVHEEEKNRKEILEKLEKHATAYRAKLKSGEIKAENQPKDNPLTRLSLKKREKKAVLFNFKGVKSLNAESLLSRVEDLKYLKNLINSNYKDDPLKFSLGNNTPKPVQNWSSNWTKEEDEKLLIGVFKYGYGSWTQIRDDPFLGITDKIFLNEVHNPVAKKSASSSDTTPTPSKKGKGITGSSKKVPGAIHLGRRVDYLLSFLRGGLNTKSPS

SEQ ID NO: 78 - protein, 1185 aa, Artificial Sequence
  SYNTHESIZED
MPKRKVSSAEGAAKEEPKRRSARLSAKPPAKVEAKPKKAAAKDKSSDKKVQTKGKRGAKGKQAEVANQETKEDLPAENGETKTEESPASDEAGEKEAKSDTGSGMARILAFDIGISSIGWAFSENDELKDCGVRIFTKVENPKTGESLALPRRLARSARKRLARRKARLNHLKHLIANEFKLNYEDYQSFDESLAKAYKGSLISPYELRFRALNELLSKQDFARVILHIAKRRGYDDIKNSDDKEKGAILKAIKQNEEKLANYQSVGEYLYKEYFQKFKENSKEFTNVRNKKESYERCIAQSFLKDELKLIFKKQREFGFSFSKKFEEEVLSVAFYKRALKDFSHLVGNCSFFTDEKRAPKNSPLAFMFVALTRIINLLNNLKNTEGILYTKDDLNALLNEVLKNGTLTYKQTKKLLGLSDDYEFKGEKGTYFIEFKKYKEFIKALGEHNLSQDDLNEIAKDITLIKDEIKLKKALAKYDLNQNQIDSLSKLEFKDHLNISFKALKLVTPLMLEGKKYDEACNELNLKVAINEDKKDFLPAFNETYYKDEVTNPVVLRAIKEYRKVLNALLKKYGKVHKINIELAREVGKNHSQRAKIEKEQNENYKAKKDAELECEKLGLKINSKNILKLRLFKEQKEFCAYSGEKIKISDLQDEKMLEIDHIYPYSRSFDDSYMNKVLVFTKQNQEKLNQTPFEAFGNDSAKWQKIEVLAKNLPTKKQKRILDKNYKDKEQKNFKDRNLNDTRYIARLVLNYTKDYLDFLPLSDDENTKLNDTQKGSKVHVEAKSGMLTSALRHTWGFSAKDRNNHLHHAIDAVIIAYANNSIVKAFSDFKKEQESNSAELYAKKISELDYKNKRKFFEPFSGFRQKVLDKIDEIFVSKPERKKPSGALHEETFRKEEEFYQSYGGKEGVLKALELGKIRKVNGKIVKNGDMFRVDIFKHKKTNKFYAVPIYTMDFALKVLPNKAVARSKKGEIKDWILMDENYEFCFSLYKDSLILIQTKDMQEPEFVYYNAFTSSTVSLIVSKHDNKFETLSKNQKILFKNANEKEVIAKSIGIQNLKVFEKYIVSALGEVTKAEFRQREDFKKPKKKRKVLEGGGGSGKGDPKKPRGKMSSYAFFVQTCREEHKKKHPDASVNFSEFSKKCSERWKTMSAKEKGKFEDMAKADKARYEREMKTYIPPKGE

SEQ ID NO: 79 - protein, 1182 aa, Artificial Sequence
  SYNTHESIZED
MPKRKVSSAEGAAKEEPKRRSARLSAKPPAKVEAKPKKAAAKDKSSDKKVQTKGKRGAKGKQAEVANQETKEDLPAENGETKTEESPASDEAGEKEAKSDTGSGMARILAFDIGISSIGWAFSENDELKDCGVRIFTKVENPKTGESLALPRRLARSARKRLARRKARLNHLKHLIANEFKLNYEDYQSFDESLAKAYKGSLISPYELRFRALNELLSKQDFARVILHIAKRRGYDDIKNSDDKEKGAILKAIKQNEEKLANYQSVGEYLYKEYFQKFKENSKEFTNVRNKKESYERCIAQSFLKDELKLIFKKQREFGFSFSKKFEEEVLSVAFYKRALKDFSHLVGNCSFFTDEKRAPKNSPLAFMFVALTRIINLLNNLKNTEGILYTKDDLNALLNEVLKNGTLTYKQTKKLLGLSDDYEFKGEKGTYFIEFKKYKEFIKALGEHNLSQDDLNEIAKDITLIKDEIKLKKALAKYDLNQNQIDSLSKLEFKDHLNISFKALKLVTPLMLEGKKYDEACNELNLKVAINEDKKDFLPAFNETYYKDEVTNPVVLRAIKEYRKVLNALLKKYGKVHKINIELAREVGKNHSQRAKIEKEQNENYKAKKDAELECEKLGLKINSKNILKLRLFKEQKEFCAYSGEKIKISDLQDEKMLEIDHIYPYSRSFDDSYMNKVLVFTKQNQEKLNQTPFEAFGNDSAKWQKIEVLAKNLPTKKQKRILDKNYKDKEQKNFKDRNLNDTRYIARLVLNYTKDYLDFLPLSDDENTKLNDTQKGSKVHVEAKSGMLTSALRHTWGFSAKDRNNHLHHAIDAVIIAYANNSIVKAFSDFKKEQESNSAELYAKKISELDYKNKRKFFEPFSGFRQKVLDKIDEIFVSKPERKKPSGALHEETFRKEEEFYQSYGGKEGVLKALELGKIRKVNGKIVKNGDMFRVDIFKHKKTNKFYAVPIYTMDFALKVLPNKAVARSKKGEIKDWILMDENYEFCFSLYKDSLILIQTKDMQEPEFVYYNAFTSSTVSLIVSKHDNKFETLSKNQKILFKNANEKEVIAKSIGIQNLKVFEKYIVSALGEVTKAEFRQREDFKKPKKKRKVLEGGGGSSTDHPKYSDMIVAAIQAEKNRAGSSRQSIQKYIKSHYKVGENADSQIKLSIKRLVTTGVLKQTKGVGASGSFRLAKSDEP